European Patent Application EP 4 159 751 A1, published April 5, 2023. Title: ANTI-KRAS-G12D T CELL RECEPTORS. Applicant: THE UNITED STATES OF AMERICA, AS REPRESENTED BY THE SECRETARY, DEPARTMENT OF HEALTH AND HUMAN SERVICES. The sequence listing filed with the application follows.

SEQUENCE LISTING (70 sequences)

SEQ ID NO: 1 - protein, 189 aa, Homo sapiens [sequence omitted]

SEQ ID NO: 2 - protein, 188 aa, Homo sapiens [sequence omitted]

SEQ ID NO: 3 - protein, 189 aa, Homo sapiens
MTEYKLVVVGADGVGKSALTIQLIQNHFVDEYDPTIEDSYRKQVVIDGETCLLDILDTAGQEEYSAMRDQYMRTGEGFLCVFAINNTKSFEDIHHYREQIKRVKDSEDVPMVLVGNKCDLPSRTVDTKQAQDLARSYGIPFIETSAKTRQRVEDAFYTLVREIRQYRLKKISKEEKTPGCVKIKKCIIM

SEQ ID NO: 4 - protein, 188 aa, Homo sapiens [sequence omitted]

SEQ ID NO: 5 - protein, 10 aa, Homo sapiens
GAGGVGKSAL

SEQ ID NO: 6 - protein, 10 aa, Homo sapiens
GADGVGKSAL

SEQ ID NO: 7 - protein, 9 aa, Homo sapiens
GAGGVGKSA

SEQ ID NO: 8 - protein, 9 aa, Homo sapiens
GADGVGKSA

SEQ ID NO: 9 - protein, 7 aa, Homo sapiens
NIATNDY

SEQ ID NO: 10 - protein, 5 aa, Homo sapiens
GYKTK

SEQ ID NO: 11 - protein, 15 aa, Homo sapiens
CLVGDMDQAGTALIF

SEQ ID NO: 12 - protein, 5 aa, Homo sapiens
SGHDT

SEQ ID NO: 13 - protein, 6 aa, Homo sapiens
YYEEEE

SEQ ID NO: 14 - protein, 15 aa, Homo sapiens
CASSLGEGRVDGYTF

SEQ ID NO: 15 - protein, 129 aa, Homo sapiens
MRQVARVIVFLTLSTLSLAKTTQPISMDSYEGQEVNITCSHNNIATNDYITWYQQFPSQGPRFIIQGYKTKVTNEVASLFIPADRKSSTLSLPRVSLSDTAVYYCLVGDMDQAGTALIFGKGTTLSVSS

SEQ ID NO: 16 - protein, 133 aa, Homo sapiens
MGPGLLCWALLCLLGAGLVDAGVTQSPTHLIKTRGQQVTLRCSPKSGHDTVSWYQQALGQGPQFIFQYYEEEERQRGNFPDRFSGHQFPNYSSELNVNALLLGDSALYLCASSLGEGRVDGYTFGSGTRLTVV

SEQ ID NO: 17 - protein, 7 aa, Homo sapiens
NIATNDY

SEQ ID NO: 18 - protein, 5 aa, Homo sapiens
GYKTK

SEQ ID NO: 19 - protein, 15 aa, Homo sapiens
CLVGDMDQAGTALIF

SEQ ID NO: 20 - protein, 5 aa, Homo sapiens
SGHDT

SEQ ID NO: 21 - protein, 6 aa, Homo sapiens
YYEEEE

SEQ ID NO: 22 - protein, 15 aa, Homo sapiens
CASSLGRASNQPQHF

SEQ ID NO: 23 - protein, 129 aa, Homo sapiens; identical to SEQ ID NO: 15

SEQ ID NO: 24 - protein, 133 aa, Homo sapiens
MGPGLLCWALLCLLGAGLVDAGVTQSPTHLIKTRGQQVTLRCSPKSGHDTVSWYQQALGQGPQFIFQYYEEEERQRGNFPDRFSGHQFPNYSSELNVNALLLGDSALYLCASSLGRASNQPQHFGDGTRLSIL

SEQ ID NO: 25 - protein, 7 aa, Homo sapiens
NIATNDY

SEQ ID NO: 26 - protein, 5 aa, Homo sapiens
GYKTK

SEQ ID NO: 27 - protein, 15 aa, Homo sapiens
CLVGDRDQAGTALIF

SEQ ID NO: 28 - protein, 5 aa, Homo sapiens
SGHDT

SEQ ID NO: 29 - protein, 6 aa, Homo sapiens
YYEEEE

SEQ ID NO: 30 - protein, 15 aa, Homo sapiens
CASSFGQSSTYGYTF

SEQ ID NO: 31 - protein, 129 aa, Homo sapiens
MRQVARVIVFLTLSTLSLAKTTQPISMDSYEGQEVNITCSHNNIATNDYITWYQQFPSQGPRFIIQGYKTKVTNEVASLFIPADRKSSTLSLPRVSLSDTAVYYCLVGDRDQAGTALIFGKGTTLSVSS

SEQ ID NO: 32 - protein, 133 aa, Homo sapiens
MGPGLLCWALLCLLGAGLVDAGVTQSPTHLIKTRGQQVTLRCSPKSGHDTVSWYQQALGQGPQFIFQYYEEEERQRGNFPDRFSGHQFPNYSSELNVNALLLGDSALYLCASSFGQSSTYGYTFGSGTRLTVV

SEQ ID NO: 33 - protein, 6 aa, Homo sapiens
DRGSQS

SEQ ID NO: 34 - protein, 6 aa, Homo sapiens
IYSNGD

SEQ ID NO: 35 - protein, 13 aa, Homo sapiens
CAAAMDSSYKLIF

SEQ ID NO: 36 - protein, 5 aa, Homo sapiens
WSHSY

SEQ ID NO: 37 - protein, 6 aa, Homo sapiens
SAAADI

SEQ ID NO: 38 - protein, 12 aa, Homo sapiens
CASSDPGTEAFF

SEQ ID NO: 39 - protein, 132 aa, Homo sapiens
MKSLRVLLVILWLQLSWVWSQQKEVEQNSGPLSVPEGAIASLNCTYSDRGSQSFFWYRQYSGKSPELIMFIYSNGDKEDGRFTAQLNKASQYVSLLIRDSQPSDSATYLCAAAMDSSYKLIFGSGTRLLVRP

SEQ ID NO: 40 - protein, 130 aa, Homo sapiens
MGTRLFFYVALCLLWAGHRDAGITQSPRYKITETGRQVTLMCHQTWSHSYMFWYRQDLGHGLRLIYYSAAADITDKGEVPDGYVVSRSKTENFPLTLESATRSQTSVYFCASSDPGTEAFFGQGTRLTVV

SEQ ID NO: 41 - protein, 141 aa, Homo sapiens
  misc_feature (1)..(1): Xaa can be any naturally occurring amino acid
XIQNPDPAVYQLRDSKSSDKSVCLFTDFDSQTNVSQSKDSDVYITDKTVLDMRSMDFKSNSAVAWSNKSDFACANAFNNSIIPEDTFFPSPESSCDVKLVEKSFETDTNLNFQNLSVIGFRILLLKVAGFNLLMTLRLWSS

SEQ ID NO: 42 - protein, 177 aa, Homo sapiens
EDLNKVFPPEVAVFEPSEAEISHTQKATLVCLATGFFPDHVELSWWVNGKEVHSGVSTDPQPLKEQPALNDSRYCLSSRLRVSATFWQNPRNHFRCQVQFYGLSENDEWTQDRAKPVTQIVSAEAWGRADCGFTSVSYQQGVLSATILYEILLGKATLYAVLVSALVLMAMVKRKDF

SEQ ID NO: 43 - protein, 179 aa, Homo sapiens
EDLKNVFPPEVAVFEPSEAEISHTQKATLVCLATGFYPDHVELSWWVNGKEVHSGVSTDPQPLKEQPALNDSRYCLSSRLRVSATFWQNPRNHFRCQVQFYGLSENDEWTQDRAKPVTQIVSAEAWGRADCGFTSESYQQGVLSATILYEILLGKATLYAVLVSALVLMAMVKRKDSRG

SEQ ID NO: 44 - protein, 137 aa, Mus musculus
DIQNPEPAVYQLKDPRSQDSTLCLFTDFDSQINVPKTMESGTFITDKTVLDMKAMDSKSNGAIAWSNQTSFTCQDIFKETNATYPSSDVPCDATLTEKSFETDMNLNFQNLSVMGLRILLLKVAGFNLLMTLRLWSS

SEQ ID NO: 45 - protein, 173 aa, Mus musculus
EDLRNVTPPKVSLFEPSKAEIANKQKATLVCLARGFFPDHVELSWWVNGKEVHSGVSTDPQAYKESNYSYCLSSRLRVSATFWHNPRNHFRCQVQFHGLSEEDKWPEGSPKPVTQNISAEAWGRADCGITSASYQQGVLSATILYEILLGKATLYAVLVSTLVVMAMVKRKNS

SEQ ID NO: 46 - protein, 137 aa, Artificial Sequence
  Synthetic
  MISC_FEATURE (48)..(48): Xaa is Thr or Cys
  MISC_FEATURE (112)..(112): Xaa is Ser, Ala, Val, Leu, Ile, Pro, Phe, Met, or Trp
  MISC_FEATURE (114)..(114): Xaa is Met, Ala, Val, Leu, Ile, Pro, Phe, or Trp
  MISC_FEATURE (115)..(115): Xaa is Gly, Ala, Val, Leu, Ile, Pro, Phe, Met, or Trp
DIQNPEPAVYQLKDPRSQDSTLCLFTDFDSQINVPKTMESGTFITDKXVLDMKAMDSKSNGAIAWSNQTSFTCQDIFKETNATYPSSDVPCDATLTEKSFETDMNLNFQNLXVXXLRILLLKVAGFNLLMTLRLWSS

SEQ ID NO: 47 - protein, 173 aa, Artificial Sequence
  Synthetic
  MISC_FEATURE (57)..(57): Xaa is Ser or Cys
EDLRNVTPPKVSLFEPSKAEIANKQKATLVCLARGFFPDHVELSWWVNGKEVHSGVXTDPQAYKESNYSYCLSSRLRVSATFWHNPRNHFRCQVQFHGLSEEDKWPEGSPKPVTQNISAEAWGRADCGITSASYQQGVLSATILYEILLGKATLYAVLVSTLVVMAMVKRKNS

SEQ ID NO: 48 - protein, 137 aa, Artificial Sequence
  Synthetic
DIQNPEPAVYQLKDPRSQDSTLCLFTDFDSQINVPKTMESGTFITDKCVLDMKAMDSKSNGAIAWSNQTSFTCQDIFKETNATYPSSDVPCDATLTEKSFETDMNLNFQNLLVIVLRILLLKVAGFNLLMTLRLWSS

SEQ ID NO: 49 - protein, 173 aa, Artificial Sequence
  Synthetic
EDLRNVTPPKVSLFEPSKAEIANKQKATLVCLARGFFPDHVELSWWVNGKEVHSGVCTDPQAYKESNYSYCLSSRLRVSATFWHNPRNHFRCQVQFHGLSEEDKWPEGSPKPVTQNISAEAWGRADCGITSASYQQGVLSATILYEILLGKATLYAVLVSTLVVMAMVKRKNS

SEQ ID NO: 50 - protein, 266 aa, Artificial Sequence
  Synthetic
MRQVARVIVFLTLSTLSLAKTTQPISMDSYEGQEVNITCSHNNIATNDYITWYQQFPSQGPRFIIQGYKTKVTNEVASLFIPADRKSSTLSLPRVSLSDTAVYYCLVGDMDQAGTALIFGKGTTLSVSSDIQNPEPAVYQLKDPRSQDSTLCLFTDFDSQINVPKTMESGTFITDKCVLDMKAMDSKSNGAIAWSNQTSFTCQDIFKETNATYPSSDVPCDATLTEKSFETDMNLNFQNLLVIVLRILLLKVAGFNLLMTLRLWSS

SEQ ID NO: 51 - protein, 306 aa, Artificial Sequence
  Synthetic
MGPGLLCWALLCLLGAGLVDAGVTQSPTHLIKTRGQQVTLRCSPKSGHDTVSWYQQALGQGPQFIFQYYEEEERQRGNFPDRFSGHQFPNYSSELNVNALLLGDSALYLCASSLGEGRVDGYTFGSGTRLTVVEDLRNVTPPKVSLFEPSKAEIANKQKATLVCLARGFFPDHVELSWWVNGKEVHSGVCTDPQAYKESNYSYCLSSRLRVSATFWHNPRNHFRCQVQFHGLSEEDKWPEGSPKPVTQNISAEAWGRADCGITSASYQQGVLSATILYEILLGKATLYAVLVSTLVVMAMVKRKNS

SEQ ID NO: 52 - protein, 266 aa, Artificial Sequence; identical to SEQ ID NO: 50
  Synthetic

SEQ ID NO: 53 - protein, 306 aa, Artificial Sequence
  Synthetic
MGPGLLCWALLCLLGAGLVDAGVTQSPTHLIKTRGQQVTLRCSPKSGHDTVSWYQQALGQGPQFIFQYYEEEERQRGNFPDRFSGHQFPNYSSELNVNALLLGDSALYLCASSLGRASNQPQHFGDGTRLSILEDLRNVTPPKVSLFEPSKAEIANKQKATLVCLARGFFPDHVELSWWVNGKEVHSGVCTDPQAYKESNYSYCLSSRLRVSATFWHNPRNHFRCQVQFHGLSEEDKWPEGSPKPVTQNISAEAWGRADCGITSASYQQGVLSATILYEILLGKATLYAVLVSTLVVMAMVKRKNS

SEQ ID NO: 54 - protein, 266 aa, Artificial Sequence
  Synthetic
MRQVARVIVFLTLSTLSLAKTTQPISMDSYEGQEVNITCSHNNIATNDYITWYQQFPSQGPRFIIQGYKTKVTNEVASLFIPADRKSSTLSLPRVSLSDTAVYYCLVGDRDQAGTALIFGKGTTLSVSSDIQNPEPAVYQLKDPRSQDSTLCLFTDFDSQINVPKTMESGTFITDKCVLDMKAMDSKSNGAIAWSNQTSFTCQDIFKETNATYPSSDVPCDATLTEKSFETDMNLNFQNLLVIVLRILLLKVAGFNLLMTLRLWSS

SEQ ID NO: 55 - protein, 306 aa, Artificial Sequence
  Synthetic
MGPGLLCWALLCLLGAGLVDAGVTQSPTHLIKTRGQQVTLRCSPKSGHDTVSWYQQALGQGPQFIFQYYEEEERQRGNFPDRFSGHQFPNYSSELNVNALLLGDSALYLCASSFGQSSTYGYTFGSGTRLTVVEDLRNVTPPKVSLFEPSKAEIANKQKATLVCLARGFFPDHVELSWWVNGKEVHSGVCTDPQAYKESNYSYCLSSRLRVSATFWHNPRNHFRCQVQFHGLSEEDKWPEGSPKPVTQNISAEAWGRADCGITSASYQQGVLSATILYEILLGKATLYAVLVSTLVVMAMVKRKNS

SEQ ID NO: 56 - protein, 269 aa, Artificial Sequence
  Synthetic
MKSLRVLLVILWLQLSWVWSQQKEVEQNSGPLSVPEGAIASLNCTYSDRGSQSFFWYRQYSGKSPELIMFIYSNGDKEDGRFTAQLNKASQYVSLLIRDSQPSDSATYLCAAAMDSSYKLIFGSGTRLLVRPDIQNPEPAVYQLKDPRSQDSTLCLFTDFDSQINVPKTMESGTFITDKCVLDMKAMDSKSNGAIAWSNQTSFTCQDIFKETNATYPSSDVPCDATLTEKSFETDMNLNFQNLLVIVLRILLLKVAGFNLLMTLRLWSS

SEQ ID NO: 57 - protein, 303 aa, Artificial Sequence
  Synthetic
MGTRLFFYVALCLLWAGHRDAGITQSPRYKITETGRQVTLMCHQTWSHSYMFWYRQDLGHGLRLIYYSAAADITDKGEVPDGYVVSRSKTENFPLTLESATRSQTSVYFCASSDPGTEAFFGQGTRLTVVEDLRNVTPPKVSLFEPSKAEIANKQKATLVCLARGFFPDHVELSWWVNGKEVHSGVCTDPQAYKESNYSYCLSSRLRVSATFWHNPRNHFRCQVQFHGLSEEDKWPEGSPKPVTQNISAEAWGRADCGITSASYQQGVLSATILYEILLGKATLYAVLVSTLVVMAMVKRKNS

SEQ ID NO: 58 - protein, 27 aa, Artificial Sequence
  Synthetic
RAKRSGSGATNFSLLKQAGDVEENPGP

SEQ ID NO: 59 - DNA, 27 bp, Artificial Sequence
  Synthetic
gccacagcactgttgctcttgaagtcc

SEQ ID NO: 60 - DNA, 24 bp, Artificial Sequence
  Synthetic
caggcagtatctggagtcattgag

SEQ ID NO: 61 - protein, 24 aa, Artificial Sequence
  Synthetic
MTEYKLVVVGAGGVGKSALTIQLI

SEQ ID NO: 62 - protein, 24 aa, Artificial Sequence
  Synthetic
MTEYKLVVVGADGVGKSALTIQLI

SEQ ID NO: 63 - DNA, 388 bp, Homo sapiens
atgaggcaagtggcgagagtgatcgtgttcctgaccctgagtactttgagccttgctaagaccacccagcccatctccatggactcatatgaaggacaagaagtgaacataacctgtagccacaacaacattgctacaaatgattatatcacgtggtaccaacagtttcccagccaaggaccacgatttattattcaaggatacaagacaaaagttacaaacgaagtggcctccctgtttatccctgccgacagaaagtccagcactctgagcctgccccgggtttccctgagcgacactgctgtgtactactgcctcgtgggtgacatggaccaggcaggaactgctctgatctttgggaagggaaccaccttatcagtgagttcca

SEQ ID NO: 64 - DNA, 400 bp, Homo sapiens
atgggccccgggctcctctgctgggcactgctttgtctcctgggagcaggcttagtggacgctggagtcacccaaagtcccacacacctgatcaaaacgagaggacagcaagtgactctgagatgctctcctaagtctgggcatgacactgtgtcctggtaccaacaggccctgggtcaggggccccagtttatctttcagtattatgaggaggaagagagacagagaggcaacttccctgatcgattctcaggtcaccagttccctaactatagctctgagctgaatgtgaacgccttgttgctgggggactcggccctctatctctgtgccagcagcttgggtgagggaagagtggacggctacaccttcggttcggggaccaggttaaccgttgtag

SEQ ID NO: 65 - DNA, 387 bp, Artificial Sequence
  Synthetic
atgcgccaggtggctcgcgtaatcgtgtttctgactctgagcactctgtcactcgccaagacgacccagcccatttcaatggactcatacgaaggtcaggaggtgaatatcacatgctcccacaataacattgctacaaacgattacattacatggtatcaacagtttccctctcaagggcctcgattcataatacaagggtataagaccaaagttacgaatgaggtcgcatccctctttattcccgccgaccggaagagttctactctttccctgcctagggtgagcctgagtgatactgctgtttactactgcctggttggagacatggaccaggcgggaactgccctcatattcggcaagggcacgacactctctgtgtcatct

SEQ ID NO: 66 - DNA, 399 bp, Artificial Sequence
  Synthetic
atggggccaggcctgctttgctgggcgctgctgtgcctcctgggtgccggtttggtggacgctggtgtaactcagtccccaacacatctgatcaagacacgcggccagcaggttacactgcgctgttcacccaagagtgggcacgatacagtttcctggtaccagcaagctctgggtcaaggacctcagtttatattccaatattacgaagaggaggagcgccagcgcggaaatttcccagacagattctccgggcaccagtttcccaactactcatctgagctgaacgttaacgccctgctgctgggagactccgctctctacctgtgcgcatctagcctcgggagggctagtaaccagccccagcacttcggcgacggaaccaggctgtctattctg

SEQ ID NO: 67 - DNA, 388 bp, Homo sapiens
atgaggcaagtggcgagagtgatcgtgttcctgaccctgagtactttgagccttgctaagaccacccagcccatctccatggactcatatgaaggacaagaagtgaacataacctgtagccacaacaacattgctacaaatgattatatcacgtggtaccaacagtttcccagccaaggaccacgatttattattcaaggatacaagacaaaagttacaaacgaagtggcctccctgtttatccctgccgacagaaagtccagcactctgagcctgccccgggtttccctgagcgacactgctgtgtactactgcctcgtgggtgacagggaccaggcaggaactgctctgatctttgggaagggaaccaccttatcagtgagttcca

SEQ ID NO: 68 - DNA, 400 bp, Homo sapiens
atgggccccgggctcctctgctgggcactgctttgtctcctgggagcaggcttagtggacgctggagtcacccaaagtcccacacacctgatcaaaacgagaggacagcaagtgactctgagatgctctcctaagtctgggcatgacactgtgtcctggtaccaacaggccctgggtcaggggccccagtttatctttcagtattatgaggaggaagagagacagagaggcaacttccctgatcgattctcaggtcaccagttccctaactatagctctgagctgaatgtgaacgccttgttgctgggggactcggccctctatctctgtgccagcagctttggacagtcaagcacatatggctacaccttcggttcggggaccaggttaaccgttgtag

SEQ ID NO: 69 - DNA, 397 bp, Homo sapiens
atgaaatccttgagagttttactagtgatcctgtggcttcagttgagctgggtttggagccaacagaaggaggtggagcagaattctggacccctcagtgttccagagggagccattgcctctctcaactgcacttacagtgaccgaggttcccagtccttcttctggtacagacaatattctgggaaaagccctgagttgataatgttcatatactccaatggtgacaaagaagatggaaggtttacagcacagctcaataaagccagccagtatgtttctctgctcatcagagactcccagcccagtgattcagccacctacctctgtgccgcggcgatggatagcagctataaattgatcttcgggagtgggaccagactgctggtcaggcctg

SEQ ID NO: 70 - DNA, 391 bp, Homo sapiens
atgggcaccaggctcttcttctatgtggccctttgtctgctgtgggcaggacacagggatgctggaatcacccagagcccaagatacaagatcacagagacaggaaggcaggtgaccttgatgtgtcaccagacttggagccacagctatatgttctggtatcgacaagacctgggacatgggctgaggctgatctattactcagcagctgctgatattacagataaaggagaagtccccgatggctatgttgtctccagatccaagacagagaatttccccctcactctggagtcagctacccgctcccagacatctgtgtatttctgcgccagcagtgaccccggcactgaagctttctttggacaaggcaccagactcacagttgtag